European Patent Application EP 4 663 752 A1, published December 17, 2025. Title: HIGHLY ACTIVE TRANSPOSASE PROTEIN OF TRANSPOSON SYSTEM, AND USE THEREOF. Applicant: NEOGENTC CORP. Application EP 24750627.2, filed February 2, 2024. The sequence listing filed with the application follows.

SEQUENCE LISTING (23 sequences)

SEQ ID NO: 1 - DNA, 1719 bp, synthetic construct
  source 1..1719: mol_type = other DNA
gcgcaacactcagattactccgacgatgaattttgtgctgacaaactgtccaattattcatgcgatagcgacctcgaaaacgcttccacgtctgatgaagatagcagcgatgatgaagtaatggtgaggcctcgcaccctccgccgtcgccgcatcagctcttcgagctctgattctgaatccgatattgagggtggccgcgaggagtggtcccacgtagacaatccgccggtgctggaggacttcctaggccaccaaggtctgaacactgacgcagtaatcaacaatatcgaagatgcagttaaactgtttatcggtgacgatttcttcgagtttctggtggaggaatctaaccggtactataaccagaatcgtaataacttcaagctctctaaaaagtctctgaagtggaaggacatcacccctcaggagatgaaaaagttcctcggtctgatcgttctgatgggccaagttcgcaaggatcgtcgtgacgactattggactaccgaaccgtggacggaaactccatactttggcaagaccatgactcgtgaccgtttccgtcagatctggaaggcctggcacttcaataacaacgctgacattgtcaacgagtctgatcgtctgtgtaaggttcgccctgtgctggattacttcgttccaaaattcattaacatttacaaaccacatcagcagctgtccctggatgagggcatcgtgccgtggcgcggccgcctgttcttccgtgtctataatgctggcaagattgtgaagtacggtatcctggttcgcctgctgtgcgaaagcgacactggctacatctgtaacatggagatctactgcggcgagggcaaacgtctcctcgaaactatccagaccgtcgtgtctccatacacggattcctggtatcatatttacatggataactattataacagcgtggctaactgtgaagctctgatgaaaaataagttccgtatttgcggtactatccgtaagaatcgtggaattccgaaagatttccagaccatctccctgaaaaagggtgaaactaagttcattcgcaaaaacgacatcctcctgcaagtctggcagtctaaaaagcctgtatatctgatctcatctattcacagcgctgaaatggaagaatctcagaacattgatcgcacctccaagaaaaagatcgtcaaaccgaatgcattgattgattacaacaagcacatgaagggcgttgatcgtgctgaccagtacctgtcttattactctatcctgcgccgtactgtgaagtggactaaacgtctcgctatgtacatgattaattgtgcgctgttcaattcttacgctgtgtataaaagcgtgcgtcagcgcaaaatgggctttaaaatgttcctgaagcagacggctattcactggctgaccgacgatattccggaagatatggacattgtcccggatctccagccggtaccgagcaccagcggtatgcgtgctaaacctccgactagtgatccgccttgccgtctgtctatggatatgcgtaagcataccctgcaggcaattgtgggctctggcaaaaagaaaaatatcctgcgtcgttgccgcgtatgctctgtacacaaactgcgttctgagactcgttatatgtgtaaattttgcaatattccactccacaagggtgcgtgcttcgagaagtaccatacgctgaagaactattctaga

SEQ ID NO: 2 - DNA, 1719 bp, synthetic construct
  source 1..1719: mol_type = other DNA
gcccagcactccgactactccgacgacgagttctgtgccgacaagttgagcaactattcatgcgacagcgatctggagaacgcttccacctcggatgaggacagctcggacgacgaggtgatggtgcggcccaggacccttcgccgccggcggatctcctcctcttcttcagattccgaaagcgatattgagggcggtagggaggagtggtctcacgtagacaaccccccggttctggaggacttcctgggccaccagggcctgaacacggacgctgtgatcaataacattgaggatgctgtaaagctgttcatcggtgatgactttttcgagttcttggtggaggagtcgaatcgctactacaaccagaaccgcaacaacttcaaactatcaaagaagagcctgaaatggaaggacatcacccctcaggagatgaagaagttccttggtctcatcgtgctcatgggccaggtgcggaaagaccgcagggacgattattggaccacagaaccgtggacggagaccccctatttcgggaaaacaatgacgcgcgaccgcttccggcaaatttggaaggcctggcactttaacaacaacgcggacatcgtcaatgagagcgaccgcctctgtaaggtgcgccccgtcctggactacttcgtccctaagttcattaacatctacaagccccaccagcagctgtccttggatgagggcatcgtgccgtggagaggacgcctgtttttccgcgtgtacaatgcgggcaagattgtgaagtacggcatcctggtgcgcctgctgtgcgagtccgacaccggctacatctgcaacatggagatctattgcggggaggggaagcggctgctggagactatccagacggtggtgtccccatacaccgacagttggtaccatatatacatggataactactacaactccgtggccaattgcgaggccctgatgaaaaacaagttccgtatctgtggcaccattcgcaaaaaccgaggcatccctaaagacttccagaccatctctctgaagaaaggggagaccaagttcatccgcaagaacgacatcttactgcaggtctggcaaagtaagaagcccgtttacctaatctcgtccattcattctgcggagatggaagagtctcagaatattgaccgcacttctaagaagaagatcgttaagcctaacgcgctcattgactacaacaagcacatgaaaggtgtcgatcgcgcagaccagtacctctcgtattacagcatcctgcgtcgtaccgtgaaatggaccaagagattggccatgtatatgatcaactgcgccctgttcaacagctacgcggtgtacaagtcggtgcgccagcgcaagatgggctttaaaatgttcctgaagcagactgctatccactggctcactgatgacatacctgaagacatggatatcgtccccgacctgcagccggtgccctctacatccggaatgcgtgctaagccaccaacctccgacccgccatgtcgtctttccatggacatgagaaagcacactcttcaggccatcgtgggctccggcaagaagaagaatatcttacgccggtgccgagtctgtagcgtccacaagctgcgctccgagacccgctacatgtgcaagttttgtaacatccccctgcacaagggagcatgctttgagaagtaccataccctgaagaactacagccgt

SEQ ID NO: 3 - DNA, 1719 bp, synthetic construct
  source 1..1719: mol_type = other DNA
gcccagcatagcgattattctgatgacgagttttgcgctgataagctgagcaactactcctgcgactccgacctggaaaacgcctctaccagcgatgaagactctagcgacgatgaagtgatggtgagacctagaacactgagaaggcggagaatctcttcctcttccagcgactccgagagcgacatcgagggaggccgcgaggaatggagccacgtggacaatcctcctgtgctggaagattttctgggccaccagggcctgaacaccgacgccgtgatcaacaatatcgaggatgctgtgaaactgttcatcggtgacgacttcttcgagttcctggttgaggaatctaatagatactacaaccagaaccggaacaacttcaaactctccaagaagagcctgaagtggaaggacatcacccctcaggagatgaagaaattcctgggactgatcgtgctgatgggccaggttcgcaaagacagacgggatgactactggacaaccgaaccttggaccgagacaccttacttcggcaagaccatgaccagagaccgatttagacaaatctggaaggcctggcacttcaacaacaatgctgacatcgtgaacgagtctgatagactgtgcaaggtgcggcctgtgctggactatttcgtgcctaagttcatcaacatctacaagccccaccagcagctgtctctggacgagggcatcgtgccctggcggggcagactgttcttcagagtgtacaacgccggcaagatcgtgaagtacggcattctggtgcggctactgtgcgagagcgacaccggctacatctgcaacatggaaatctactgcggcgagggcaaacggctcctggaaaccatccagaccgtggtgtccccttatacagacagctggtatcacatctacatggataactactacaatagcgtggccaactgcgaggccctgatgaagaacaagttccggatctgtggcaccatcagaaagaaccggggcattcctaaggacttccagactatcagcctgaagaagggcgagacaaagtttattaggaagaacgacatcctgctgcaagtgtggcagagcaaaaaacccgtttacctgatcagcagcatccacagcgccgagatggaagagtctcagaacatcgatagaaccagcaagaaaaagatcgtgaaaccaaacgcactgatcgactacaacaagcacatgaagggcgtggatagagccgatcagtacctgagctactacagcatcctgagaaggacagtcaagtggaccaagagacttgctatgtacatgatcaactgtgccctgttcaacagctacgccgtgtacaagagcgtgcggcagagaaagatgggatttaagatgttcctgaaacagacagccatccactggctgaccgacgacatccctgaggacatggacatcgtccccgacctgcaacccgtgcctagcaccagcggcatgcgggccaagccacctaccagtgaccccccatgtagactgagcatggacatgagaaaacatacactgcaagccatcgtcggcagcggaaagaaaaagaatatcctgagaagatgcagagtgtgcagcgtgcacaagctgagaagcgagactcggtacatgtgcaagttctgtaatatccccctgcacaagggagcctgcttcgagaagtaccacaccctgaagaactacagcaga

SEQ ID NO: 4 - DNA, 21 bp, synthetic construct
  source 1..21: mol_type = other DNA
cccaagaagaagaggaaagtc

SEQ ID NO: 5 - DNA, 21 bp, synthetic construct
  source 1..21: mol_type = other DNA
ccaaagaagaagcgtaaggta

SEQ ID NO: 6 - DNA, 21 bp, synthetic construct
  source 1..21: mol_type = other DNA
ccaaagaaaaagaggaaagtc

SEQ ID NO: 7 - DNA, 21 bp, synthetic construct
  source 1..21: mol_type = other DNA
cctaaaaagaaacgaaaggtt

SEQ ID NO: 8 - DNA, 21 bp, synthetic construct
  source 1..21: mol_type = other DNA
ccaaaaaagaagagaaaggta

SEQ ID NO: 9 - DNA, 21 bp, synthetic construct
  source 1..21: mol_type = other DNA
cccaaaaagaagcgcaaggtg

SEQ ID NO: 10 - DNA, 27 bp, synthetic construct
  source 1..27: mol_type = other DNA
cctgctgccaagagggtcaagttggac

SEQ ID NO: 11 - DNA, 27 bp, synthetic construct
  source 1..27: mol_type = other DNA
cccgcggctaagcgcgtgaagctggac

SEQ ID NO: 12 - RNA, 1725 nt, synthetic construct
  source 1..1725: mol_type = other RNA
atggcccagcatagcgattattctgatgacgagttttgcgctgataagctgagcaactactcctgcgactccgacctggaaaacgcctctaccagcgatgaagactctagcgacgatgaagtgatggtgagacctagaacactgagaaggcggagaatctcttcctcttccagcgactccgagagcgacatcgagggaggccgcgaggaatggagccacgtggacaatcctcctgtgctggaagattttctgggccaccagggcctgaacaccgacgccgtgatcaacaatatcgaggatgctgtgaaactgttcatcggtgacgacttcttcgagttcctggttgaggaatctaatagatactacaaccagaaccggaacaacttcaaactctccaagaagagcctgaagtggaaggacatcacccctcaggagatgaagaaattcctgggactgatcgtgctgatgggccaggttcgcaaagacagacgggatgactactggacaaccgaaccttggaccgagacaccttacttcggcaagaccatgaccagagaccgatttagacaaatctggaaggcctggcacttcaacaacaatgctgacatcgtgaacgagtctgatagactgtgcaaggtgcggcctgtgctggactatttcgtgcctaagttcatcaacatctacaagccccaccagcagctgtctctggacgagggcatcgtgccctggcggggcagactgttcttcagagtgtacaacgccggcaagatcgtgaagtacggcattctggtgcggctactgtgcgagagcgacaccggctacatctgcaacatggaaatctactgcggcgagggcaaacggctcctggaaaccatccagaccgtggtgtccccttatacagacagctggtatcacatctacatggataactactacaatagcgtggccaactgcgaggccctgatgaagaacaagttccggatctgtggcaccatcagaaagaaccggggcattcctaaggacttccagactatcagcctgaagaagggcgagacaaagtttattaggaagaacgacatcctgctgcaagtgtggcagagcaaaaaacccgtttacctgatcagcagcatccacagcgccgagatggaagagtctcagaacatcgatagaaccagcaagaaaaagatcgtgaaaccaaacgcactgatcgactacaacaagcacatgaagggcgtggatagagccgatcagtacctgagctactacagcatcctgagaaggacagtcaagtggaccaagagacttgctatgtacatgatcaactgtgccctgttcaacagctacgccgtgtacaagagcgtgcggcagagaaagatgggatttaagatgttcctgaaacagacagccatccactggctgaccgacgacatccctgaggacatggacatcgtccccgacctgcaacccgtgcctagcaccagcggcatgcgggccaagccacctaccagtgaccccccatgtagactgagcatggacatgagaaaacatacactgcaagccatcgtcggcagcggaaagaaaaagaatatcctgagaagatgcagagtgtgcagcgtgcacaagctgagaagcgagactcggtacatgtgcaagttctgtaatatccccctgcacaagggagcctgcttcgagaagtaccacaccctgaagaactacagcagatga

SEQ ID NO: 13 - protein, 574 aa, synthetic construct
MAQHSDYSDDEFCADKLSNYSCDSDLENASTSDEDSSDDEVMVRPRTLRRRRISSSSSDSESDIEGGREEWSHVDNPPVLEDFLGHQGLNTDAVINNIEDAVKLFIGDDFFEFLVEESNRYYNQNRNNFKLSKKSLKWKDITPQEMKKFLGLIVLMGQVRKDRRDDYWTTEPWTETPYFGKTMTRDRFRQIWKAWHFNNNADIVNESDRLCKVRPVLDYFVPKFINIYKPHQQLSLDEGIVPWRGRLFFRVYNAGKIVKYGILVRLLCESDTGYICNMEIYCGEGKRLLETIQTVVSPYTDSWYHIYMDNYYNSVANCEALMKNKFRICGTIRKNRGIPKDFQTISLKKGETKFIRKNDILLQVWQSKKPVYLISSIHSAEMEESQNIDRTSKKKIVKPNALIDYNKHMKGVDRADQYLSYYSILRRTVKWTKRLAMYMINCALFNSYAVYKSVRQRKMGFKMFLKQTAIHWLTDDIPEDMDIVPDLQPVPSTSGMRAKPPTSDPPCRLSMDMRKHTLQAIVGSGKKKNILRRCRVCSVHKLRSETRYMCKFCNIPLHKGACFEKYHTLKNYSR

SEQ ID NO: 14 - DNA, 6632 bp, synthetic construct
  source 1..6632: mol_type = other DNA
agcgttaatattttgttaaaattcgcgttaaatttttgttaaatcagctcattttttaaccaataggccgaaatcggcaaaatcccttataaatcaaaagaatagaccgagatagggttgagtgttgttccagtttggaacaagagtccactattaaagaacgtggactccaacgtcaaagggcgaaaaaccgtctatcagggcgatggcccactacgtgaaccatcaccctaatcaagttttttggggtcgaggtgccgtaaagcactaaatcggaaccctaaagggagcccccgatttagagcttgacggggaaagccggcgaacgtggcgagaaaggaagggaagaaagcgaaaggagcgggcgctagggcgctggcaagtgtagcggtcacgctgcgcgtaaccaccacacccgccgcgcttaatgcgccgctacagggcgcgtcccattcgccattcaggctgcgcaactgttgggaagggcgatcggtgcgggcctcttcgctattacgccagctggcgaaagggggatgtgctgcaaggcgattaagttgggtaacgccagggttttcccagtcacgacgttgtaaaacgacggccagtgaattgtaatacgactcactatagggcgaattgggtaccggccatgatggccgaattaattcaagctagtcgacattgattattgactagttattaatagtaatcaattacggggtcattagttcatagcccatatatggagttccgcgttacataacttacggtaaatggcccgcctggctgaccgcccaacgacccccgcccattgacgtcaataatgacgtatgttcccatagtaacgccaatagggactttccattgacgtcaatgggtggactatttacggtaaactgcccacttggcagtacatcaagtgtatcatatgccaagtacgccccctattgacgtcaatgacggtaaatggcccgcctggcattatgcccagtacatgaccttatgggactttcctacttggcagtacatctacgtattagtcatcgctattaccatgggtcgaggtgagccccacgttctgcttcactctccccatctcccccccctccccacccccaattttgtatttatttattttttaattattttgtgcagcgatgggggcggggggggggggggcgcgcgccaggcggggcggggcggggcgaggggcggggcggggcgaggcggagaggtgcggcggcagccaatcagagcggcgcgctccgaaagtttccttttatggcgaggcggcggcggcggcggccctataaaaagcgaagcgcgcggcgggcgggagtcgctgcgttgccttcgccccgtgccccgctccgcgccgcctcgcgccgcccgccccggctctgactgaccgcgttactcccacaggtgagcgggcgggacggcccttctcctccgggctgtaattagcgcttggtttaatgacggctcgtttcttttctgtggctgcgtgaaagccttaaagggctccgggagggccctttgtgcgggggggagcggctcggggggtgcgtgcgtgtgtgtgtgcgtggggagcgccgcgtgcggcccgcgctgcccggcggctgtgagcgctgcgggcgcggcgcggggctttgtgcgctccgcgtgtgcgcgaggggagcgcggccgggggcggtgccccgcggtgcgggggggctgcgaggggaacaaaggctgcgtgcggggtgtgtgcgtgggggggtgagcagggggtgtgggcgcggcggtcgggctgtaacccccccctgcacccccctccccgagttgctgagcacggcccggcttcgggtgcggggctccgtgcggggcgtggcgcggggctcgccgtgccgggcggggggtggcggcaggtgggggtgccgggcggggcggggccgcctcgggccggggagggctcgggggaggggcgcggcggccccggagcgccggcggctgtcgaggcgcggcgagccgcagccattgccttttatggtaatcgtgcgagagggcgcagggacttcctttgtcccaaatctggcggagccgaaatctgggaggcgccgccgcaccccctctagcgggcgcgggcgaagcggtgcggcgccggcaggaaggaaatgggcggggagggccttcgtgcgtcgccgcgccgccgtccccttctccatctccagcctcggggctgccgcagggggacggctgccttcgggggggacggggcagggcggggttcggcttctggcgtgtgaccggcggctctagagcctctgctaaccatgttcatgccttcttctttttcctacagctcctgggcaacgtgctggttattgtgctgtctcatcattttggcaaagaattggatccatggcccagcactccgactactccgacgacgagttctgtgccgacaagttgagcaactattcatgcgacagcgatctggagaacgcttccacctcggatgaggacagctcggacgacgaggtgatggtgcggcccaggacccttcgccgccggcggatctcctcctcttcttcagattccgaaagcgatattgagggcggtagggaggagtggtctcacgtagacaaccccccggttctggaggacttcctgggccaccagggcctgaacacggacgctgtgatcaataacattgaggatgctgtaaagctgttcatcggtgatgactttttcgagttcttggtggaggagtcgaatcgctactacaaccagaaccgcaacaacttcaaactatcaaagaagagcctgaaatggaaggacatcacccctcaggagatgaagaagttccttggtctcatcgtgctcatgggccaggtgcggaaagaccgcagggacgattattggaccacagaaccgtggacggagaccccctatttcgggaaaacaatgacgcgcgaccgcttccggcaaatttggaaggcctggcactttaacaacaacgcggacatcgtcaatgagagcgaccgcctctgtaaggtgcgccccgtcctggactacttcgtccctaagttcattaacatctacaagccccaccagcagctgtccttggatgagggcatcgtgccgtggagaggacgcctgtttttccgcgtgtacaatgcgggcaagattgtgaagtacggcatcctggtgcgcctgctgtgcgagtccgacaccggctacatctgcaacatggagatctattgcggggaggggaagcggctgctggagactatccagacggtggtgtccccatacaccgacagttggtaccatatatacatggataactactacaactccgtggccaattgcgaggccctgatgaaaaacaagttccgtatctgtggcaccattcgcaaaaaccgaggcatccctaaagacttccagaccatctctctgaagaaaggggagaccaagttcatccgcaagaacgacatcttactgcaggtctggcaaagtaagaagcccgtttacctaatctcgtccattcattctgcggagatggaagagtctcagaatattgaccgcacttctaagaagaagatcgttaagcctaacgcgctcattgactacaacaagcacatgaaaggtgtcgatcgcgcagaccagtacctctcgtattacagcatcctgcgtcgtaccgtgaaatggaccaagagattggccatgtatatgatcaactgcgccctgttcaacagctacgcggtgtacaagtcggtgcgccagcgcaagatgggctttaaaatgttcctgaagcagactgctatccactggctcactgatgacatacctgaagacatggatatcgtccccgacctgcagccggtgccctctacatccggaatgcgtgctaagccaccaacctccgacccgccatgtcgtctttccatggacatgagaaagcacactcttcaggccatcgtgggctccggcaagaagaagaatatcttacgccggtgccgagtctgtagcgtccacaagctgcgctccgagacccgctacatgtgcaagttttgtaacatccccctgcacaagggagcatgctttgagaagtaccataccctgaagaactacagccgttgactcgagggccgctgatcagcctcgactgtgccttctagttgccagccatctgttgtttgcccctcccccgtgccttccttgaccctggaaggtgccactcccactgtcctttcctaataaaatgaggaaattgcatcgcattgtctgagtaggtgtcattctattctggggggtggggtggggcaggacagcaagggggaggattgggaagacaatagcaggcatgctggggatgcggtgggctctatggcttctgaggcggaaagaaccagctggggcttaattaagagctccagcttttgttccctttagtgagggttaatttcgagcttggcgtaatcatggtcatagctgtttcctgtgtgaaattgttatccgctcacaattccacacaacatacgagccggaagcataaagtgtaaagcctggggtgcctaatgagtgagctaactcacattaattgcgttgcgctcactgcccgctttccagtcgggaaacctgtcgtgccagctgcattaatgaatcggccaacgcgcggggagaggcggtttgcgtattgggcgctcttccgcttcctcgctcactgactcgctgcgctcggtcgttcggctgcggcgagcggtatcagctcactcaaaggcggtaatacggttatccacagaatcaggggataacgcaggaaagaacatgtgagcaaaaggccagcaaaaggccaggaaccgtaaaaaggccgcgttgctggcgtttttccataggctccgcccccctgacgagcatcacaaaaatcgacgctcaagtcagaggtggcgaaacccgacaggactataaagataccaggcgtttccccctggaagctccctcgtgcgctctcctgttccgaccctgccgcttaccggatacctgtccgcctttctcccttcgggaagcgtggcgctttctcatagctcacgctgtaggtatctcagttcggtgtaggtcgttcgctccaagctgggctgtgtgcacgaaccccccgttcagcccgaccgctgcgccttatccggtaactatcgtcttgagtccaacccggtaagacacgacttatcgccactggcagcagccactggtaacaggattagcagagcgaggtatgtaggcggtgctacagagttcttgaagtggtggcctaactacggctacactagaaggacagtatttggtatctgcgctctgctgaagccagttaccttcggaaaaagagttggtagctcttgatccggcaaacaaaccaccgctggtagcggtggtttttttgtttgcaagcagcagattacgcgcagaaaaaaaggatctcaagaagatcctttgatcttttctacggggtctgacgctcagtggaacgaaaactcacgttaagggattttggtcatgagattatcaaaaaggatcttcacctagatccttttaaattaaaaatgaagttttaaatcaatctaaagtatatatgagtaaacttggtctgacagttaccaatgcttaatcagtgaggcacctatctcagcgatctgtctatttcgttcatccatagttgcctgactccccgtcgtgtagataactacgatacgggagggcttaccatctggccccagtgctgcaatgataccgcgagacccacgctcaccggctccagatttatcagcaataaaccagccagccggaagggccgagcgcagaagtggtcctgcaactttatccgcctccatccagtctattaattgttgccgggaagctagagtaagtagttcgccagttaatagtttgcgcaacgttgttgccattgctacaggcatcgtggtgtcacgctcgtcgtttggtatggcttcattcagctccggttcccaacgatcaaggcgagttacatgatcccccatgttgtgcaaaaaagcggttagctccttcggtcctccgatcgttgtcagaagtaagttggccgcagtgttatcactcatggttatggcagcactgcataattctcttactgtcatgccatccgtaagatgcttttctgtgactggtgagtactcaaccaagtcattctgagaatagtgtatgcggcgaccgagttgctcttgcccggcgtcaatacgggataataccgcgccacatagcagaactttaaaagtgctcatcattggaaaacgttcttcggggcgaaaactctcaaggatcttaccgctgttgagatccagttcgatgtaacccactcgtgcacccaactgatcttcagcatcttttactttcaccagcgtttctgggtgagcaaaaacaggaaggcaaaatgccgcaaaaaagggaataagggcgacacggaaatgttgaatactcatactcttcctttttcaatattattgaagcatttatcagggttattgtctcatgagcggatacatatttgaatgtatttagaaaaataaacaaataggggttccgcgcacatttccccgaaaagtgccacctaaattgta

SEQ ID NO: 15 - DNA, 4646 bp, synthetic construct
  source 1..4646: mol_type = other DNA
atggcgcaggggatcaagctctgatcaagagacaggatgaggatcgtttcgcatgattgaacaagatggattgcacgcaggttctccggccgcttgggtggagaggctattcggctatgactgggcacaacagacaatcggctgctctgatgccgccgtgttccggctgtcagcgcaggggcgcccggttctttttgtcaagaccgacctgtccggtgccctgaatgaactgcaagacgaggcagcgcggctatcgtggctggccacgacgggcgttccttgcgcagctgtgctcgacgttgtcactgaagcgggaagggactggctgctattgggcgaagtgccggggcaggatctcctgtcatctcaccttgctcctgccgagaaagtatccatcatggctgatgcaatgcggcggctgcatacgcttgatccggctacctgcccattcgaccaccaagcgaaacatcgcatcgagcgagcacgtactcggatggaagccggtcttgtcgatcaggatgatctggacgaagagcatcaggggctcgcgccagccgaactgttcgccaggctcaaggcgagcatgcccgacggcgaggatctcgtcgtgacccatggcgatgcctgcttgccgaatatcatggtggaaaatggccgcttttctggattcatcgactgtggccggctgggtgtggcggaccgctatcaggacatagcgttggctacccgtgatattgctgaagagcttggcggcgaatgggctgaccgcttcctcgtgctttacggtatcgccgctcccgattcgcagcgcatcgccttctatcgccttcttgacgagttcttctgaattattaacgcttacaatttcctgatgcggtattttctccttacgcatctgtgcggtatttcacaccgcatcaggtggcacttttcggggaaatgtgcgcggaacccctatttgtttatttttctaaatacattcaaatatgtatccgctcatgagacaataaccctgataaatgcttcaataatagcacgtgctaaaacttcatttttaatttaaaaggatctaggtgaagatcctttttgataatctcatgaccaaaatcccttaacgtgagttttcgttccactgagcgtcagaccccgtagaaaagatcaaaggatcttcttgagatcctttttttctgcgcgtaatctgctgcttgcaaacaaaaaaaccaccgctaccagcggtggtttgtttgccggatcaagagctaccaactctttttccgaaggtaactggcttcagcagagcgcagataccaaatactgttcttctagtgtagccgtagttaggccaccacttcaagaactctgtagcaccgcctacatacctcgctctgctaatcctgttaccagtggctgctgccagtggcgataagtcgtgtcttaccgggttggactcaagacgatagttaccggataaggcgcagcggtcgggctgaacggggggttcgtgcacacagcccagcttggagcgaacgacctacaccgaactgagatacctacagcgtgagctatgagaaagcgccacgcttcccgaagggagaaaggcggacaggtatccggtaagcggcagggtcggaacaggagagcgcacgagggagcttccagggggaaacgcctggtatctttatagtcctgtcgggtttcgccacctctgacttgagcgtcgatttttgtgatgctcgtcaggggggcggagcctatggaaaaacgccagcaacgcggcctttttacggttcctggccttttgctggccttttgctcacatgttcttgctgcttcgcgatgtacgggccagatatacgcgttgacattgattattgactagttattaatagtaatcaattacggggtcattagttcatagcccatatatggagttccgcgttacataacttacggtaaatggcccgcctggctgaccgcccaacgacccccgcccattgacgtcaataatgacgtatgttcccatagtaacgccaatagggactttccattgacgtcaatgggtggagtatttacggtaaactgcccacttggcagtacatcaagtgtatcatatgccaagtacgccccctattgacgtcaatgacggtaaatggcccgcctggcattatgcccagtacatgaccttatgggactttcctacttggcagtacatctacgtattagtcatcgctattaccatggtgatgcggttttggcagtacatcaatgggcgtggatagcggtttgactcacggggatttccaagtctccaccccattgacgtcaatgggagtttgttttggcaccaaaatcaacgggactttccaaaatgtcgtaacaactccgccccattgacgcaaatgggcggtaggcgtgtacggtgggaggtctatataagcagagctctctggctaactagagaacccactgcttactggcttatcgaaattaatacgactcactataaggaataaactagtattcttctggtccccacagactcagagagaacccgccaccatggcccagcatagcgattattctgatgacgagttttgcgctgataagctgagcaactactcctgcgactccgacctggaaaacgcctctaccagcgatgaagactctagcgacgatgaagtgatggtgagacctagaacactgagaaggcggagaatctcttcctcttccagcgactccgagagcgacatcgagggaggccgcgaggaatggagccacgtggacaatcctcctgtgctggaagattttctgggccaccagggcctgaacaccgacgccgtgatcaacaatatcgaggatgctgtgaaactgttcatcggtgacgacttcttcgagttcctggttgaggaatctaatagatactacaaccagaaccggaacaacttcaaactctccaagaagagcctgaagtggaaggacatcacccctcaggagatgaagaaattcctgggactgatcgtgctgatgggccaggttcgcaaagacagacgggatgactactggacaaccgaaccttggaccgagacaccttacttcggcaagaccatgaccagagaccgatttagacaaatctggaaggcctggcacttcaacaacaatgctgacatcgtgaacgagtctgatagactgtgcaaggtgcggcctgtgctggactatttcgtgcctaagttcatcaacatctacaagccccaccagcagctgtctctggacgagggcatcgtgccctggcggggcagactgttcttcagagtgtacaacgccggcaagatcgtgaagtacggcattctggtgcggctactgtgcgagagcgacaccggctacatctgcaacatggaaatctactgcggcgagggcaaacggctcctggaaaccatccagaccgtggtgtccccttatacagacagctggtatcacatctacatggataactactacaatagcgtggccaactgcgaggccctgatgaagaacaagttccggatctgtggcaccatcagaaagaaccggggcattcctaaggacttccagactatcagcctgaagaagggcgagacaaagtttattaggaagaacgacatcctgctgcaagtgtggcagagcaaaaaacccgtttacctgatcagcagcatccacagcgccgagatggaagagtctcagaacatcgatagaaccagcaagaaaaagatcgtgaaaccaaacgcactgatcgactacaacaagcacatgaagggcgtggatagagccgatcagtacctgagctactacagcatcctgagaaggacagtcaagtggaccaagagacttgctatgtacatgatcaactgtgccctgttcaacagctacgccgtgtacaagagcgtgcggcagagaaagatgggatttaagatgttcctgaaacagacagccatccactggctgaccgacgacatccctgaggacatggacatcgtccccgacctgcaacccgtgcctagcaccagcggcatgcgggccaagccacctaccagtgaccccccatgtagactgagcatggacatgagaaaacatacactgcaagccatcgtcggcagcggaaagaaaaagaatatcctgagaagatgcagagtgtgcagcgtgcacaagctgagaagcgagactcggtacatgtgcaagttctgtaatatccccctgcacaagggagcctgcttcgagaagtaccacaccctgaagaactacagcagatgatgagctggagcctcggtggcctagcttcttgccccttgggcctccccccagcccctcctccccttcctgcacccgtacccccgtggtctttgaataaagtctgagtgggcggcaaaaaaaaaaaaaaaaaaaaaaaaaaaaaaaaaaaaaaaaaaaaaaaaaaaaaaaaaaaaaaaaaaaaaaaaaaaaaaaaaaaaaaaaaaaaaaaaaaaaaaaaagcttctcgagtcgacctaggatcccttctactgggcggttttatggacagcaagcgaaccggaattgccagctggggcgccctctggtaaggttgggaagccctgcaaagtaaactggatggctttcttgccgccaaggatctg

SEQ ID NO: 16 - DNA, 1740 bp, synthetic construct
  source 1..1740: mol_type = other DNA
cccaaaaagaagcgcaaggtggcccagcactccgactactccgacgacgagttctgtgccgacaagttgagcaactattcatgcgacagcgatctggagaacgcttccacctcggatgaggacagctcggacgacgaggtgatggtgcggcccaggacccttcgccgccggcggatctcctcctcttcttcagattccgaaagcgatattgagggcggtagggaggagtggtctcacgtagacaaccccccggttctggaggacttcctgggccaccagggcctgaacacggacgctgtgatcaataacattgaggatgctgtaaagctgttcatcggtgatgactttttcgagttcttggtggaggagtcgaatcgctactacaaccagaaccgcaacaacttcaaactatcaaagaagagcctgaaatggaaggacatcacccctcaggagatgaagaagttccttggtctcatcgtgctcatgggccaggtgcggaaagaccgcagggacgattattggaccacagaaccgtggacggagaccccctatttcgggaaaacaatgacgcgcgaccgcttccggcaaatttggaaggcctggcactttaacaacaacgcggacatcgtcaatgagagcgaccgcctctgtaaggtgcgccccgtcctggactacttcgtccctaagttcattaacatctacaagccccaccagcagctgtccttggatgagggcatcgtgccgtggagaggacgcctgtttttccgcgtgtacaatgcgggcaagattgtgaagtacggcatcctggtgcgcctgctgtgcgagtccgacaccggctacatctgcaacatggagatctattgcggggaggggaagcggctgctggagactatccagacggtggtgtccccatacaccgacagttggtaccatatatacatggataactactacaactccgtggccaattgcgaggccctgatgaaaaacaagttccgtatctgtggcaccattcgcaaaaaccgaggcatccctaaagacttccagaccatctctctgaagaaaggggagaccaagttcatccgcaagaacgacatcttactgcaggtctggcaaagtaagaagcccgtttacctaatctcgtccattcattctgcggagatggaagagtctcagaatattgaccgcacttctaagaagaagatcgttaagcctaacgcgctcattgactacaacaagcacatgaaaggtgtcgatcgcgcagaccagtacctctcgtattacagcatcctgcgtcgtaccgtgaaatggaccaagagattggccatgtatatgatcaactgcgccctgttcaacagctacgcggtgtacaagtcggtgcgccagcgcaagatgggctttaaaatgttcctgaagcagactgctatccactggctcactgatgacatacctgaagacatggatatcgtccccgacctgcagccggtgccctctacatccggaatgcgtgctaagccaccaacctccgacccgccatgtcgtctttccatggacatgagaaagcacactcttcaggccatcgtgggctccggcaagaagaagaatatcttacgccggtgccgagtctgtagcgtccacaagctgcgctccgagacccgctacatgtgcaagttttgtaacatccccctgcacaagggagcatgctttgagaagtaccataccctgaagaactacagccgt

SEQ ID NO: 17 - DNA, 6659 bp, synthetic construct
  source 1..6659: mol_type = other DNA
agcgttaatattttgttaaaattcgcgttaaatttttgttaaatcagctcattttttaaccaataggccgaaatcggcaaaatcccttataaatcaaaagaatagaccgagatagggttgagtgttgttccagtttggaacaagagtccactattaaagaacgtggactccaacgtcaaagggcgaaaaaccgtctatcagggcgatggcccactacgtgaaccatcaccctaatcaagttttttggggtcgaggtgccgtaaagcactaaatcggaaccctaaagggagcccccgatttagagcttgacggggaaagccggcgaacgtggcgagaaaggaagggaagaaagcgaaaggagcgggcgctagggcgctggcaagtgtagcggtcacgctgcgcgtaaccaccacacccgccgcgcttaatgcgccgctacagggcgcgtcccattcgccattcaggctgcgcaactgttgggaagggcgatcggtgcgggcctcttcgctattacgccagctggcgaaagggggatgtgctgcaaggcgattaagttgggtaacgccagggttttcccagtcacgacgttgtaaaacgacggccagtgaattgtaatacgactcactatagggcgaattgggtaccggccatgatggccgaattaattcaagctagtcgacattgattattgactagttattaatagtaatcaattacggggtcattagttcatagcccatatatggagttccgcgttacataacttacggtaaatggcccgcctggctgaccgcccaacgacccccgcccattgacgtcaataatgacgtatgttcccatagtaacgccaatagggactttccattgacgtcaatgggtggactatttacggtaaactgcccacttggcagtacatcaagtgtatcatatgccaagtacgccccctattgacgtcaatgacggtaaatggcccgcctggcattatgcccagtacatgaccttatgggactttcctacttggcagtacatctacgtattagtcatcgctattaccatgggtcgaggtgagccccacgttctgcttcactctccccatctcccccccctccccacccccaattttgtatttatttattttttaattattttgtgcagcgatgggggcggggggggggggggcgcgcgccaggcggggcggggcggggcgaggggcggggcggggcgaggcggagaggtgcggcggcagccaatcagagcggcgcgctccgaaagtttccttttatggcgaggcggcggcggcggcggccctataaaaagcgaagcgcgcggcgggcgggagtcgctgcgttgccttcgccccgtgccccgctccgcgccgcctcgcgccgcccgccccggctctgactgaccgcgttactcccacaggtgagcgggcgggacggcccttctcctccgggctgtaattagcgcttggtttaatgacggctcgtttcttttctgtggctgcgtgaaagccttaaagggctccgggagggccctttgtgcgggggggagcggctcggggggtgcgtgcgtgtgtgtgtgcgtggggagcgccgcgtgcggcccgcgctgcccggcggctgtgagcgctgcgggcgcggcgcggggctttgtgcgctccgcgtgtgcgcgaggggagcgcggccgggggcggtgccccgcggtgcgggggggctgcgaggggaacaaaggctgcgtgcggggtgtgtgcgtgggggggtgagcagggggtgtgggcgcggcggtcgggctgtaacccccccctgcacccccctccccgagttgctgagcacggcccggcttcgggtgcggggctccgtgcggggcgtggcgcggggctcgccgtgccgggcggggggtggcggcaggtgggggtgccgggcggggcggggccgcctcgggccggggagggctcgggggaggggcgcggcggccccggagcgccggcggctgtcgaggcgcggcgagccgcagccattgccttttatggtaatcgtgcgagagggcgcagggacttcctttgtcccaaatctggcggagccgaaatctgggaggcgccgccgcaccccctctagcgggcgcgggcgaagcggtgcggcgccggcaggaaggaaatgggcggggagggccttcgtgcgtcgccgcgccgccgtccccttctccatctccagcctcggggctgccgcagggggacggctgccttcgggggggacggggcagggcggggttcggcttctggcgtgtgaccggcggctctagagcctctgctaaccatgttcatgccttcttctttttcctacagctcctgggcaacgtgctggttattgtgctgtctcatcattttggcaaagaattggatccgccaccatgcccaaaaagaagcgcaaggtggcccagcactccgactactccgacgacgagttctgtgccgacaagttgagcaactattcatgcgacagcgatctggagaacgcttccacctcggatgaggacagctcggacgacgaggtgatggtgcggcccaggacccttcgccgccggcggatctcctcctcttcttcagattccgaaagcgatattgagggcggtagggaggagtggtctcacgtagacaaccccccggttctggaggacttcctgggccaccagggcctgaacacggacgctgtgatcaataacattgaggatgctgtaaagctgttcatcggtgatgactttttcgagttcttggtggaggagtcgaatcgctactacaaccagaaccgcaacaacttcaaactatcaaagaagagcctgaaatggaaggacatcacccctcaggagatgaagaagttccttggtctcatcgtgctcatgggccaggtgcggaaagaccgcagggacgattattggaccacagaaccgtggacggagaccccctatttcgggaaaacaatgacgcgcgaccgcttccggcaaatttggaaggcctggcactttaacaacaacgcggacatcgtcaatgagagcgaccgcctctgtaaggtgcgccccgtcctggactacttcgtccctaagttcattaacatctacaagccccaccagcagctgtccttggatgagggcatcgtgccgtggagaggacgcctgtttttccgcgtgtacaatgcgggcaagattgtgaagtacggcatcctggtgcgcctgctgtgcgagtccgacaccggctacatctgcaacatggagatctattgcggggaggggaagcggctgctggagactatccagacggtggtgtccccatacaccgacagttggtaccatatatacatggataactactacaactccgtggccaattgcgaggccctgatgaaaaacaagttccgtatctgtggcaccattcgcaaaaaccgaggcatccctaaagacttccagaccatctctctgaagaaaggggagaccaagttcatccgcaagaacgacatcttactgcaggtctggcaaagtaagaagcccgtttacctaatctcgtccattcattctgcggagatggaagagtctcagaatattgaccgcacttctaagaagaagatcgttaagcctaacgcgctcattgactacaacaagcacatgaaaggtgtcgatcgcgcagaccagtacctctcgtattacagcatcctgcgtcgtaccgtgaaatggaccaagagattggccatgtatatgatcaactgcgccctgttcaacagctacgcggtgtacaagtcggtgcgccagcgcaagatgggctttaaaatgttcctgaagcagactgctatccactggctcactgatgacatacctgaagacatggatatcgtccccgacctgcagccggtgccctctacatccggaatgcgtgctaagccaccaacctccgacccgccatgtcgtctttccatggacatgagaaagcacactcttcaggccatcgtgggctccggcaagaagaagaatatcttacgccggtgccgagtctgtagcgtccacaagctgcgctccgagacccgctacatgtgcaagttttgtaacatccccctgcacaagggagcatgctttgagaagtaccataccctgaagaactacagccgttgactcgagggccgctgatcagcctcgactgtgccttctagttgccagccatctgttgtttgcccctcccccgtgccttccttgaccctggaaggtgccactcccactgtcctttcctaataaaatgaggaaattgcatcgcattgtctgagtaggtgtcattctattctggggggtggggtggggcaggacagcaagggggaggattgggaagacaatagcaggcatgctggggatgcggtgggctctatggcttctgaggcggaaagaaccagctggggcttaattaagagctccagcttttgttccctttagtgagggttaatttcgagcttggcgtaatcatggtcatagctgtttcctgtgtgaaattgttatccgctcacaattccacacaacatacgagccggaagcataaagtgtaaagcctggggtgcctaatgagtgagctaactcacattaattgcgttgcgctcactgcccgctttccagtcgggaaacctgtcgtgccagctgcattaatgaatcggccaacgcgcggggagaggcggtttgcgtattgggcgctcttccgcttcctcgctcactgactcgctgcgctcggtcgttcggctgcggcgagcggtatcagctcactcaaaggcggtaatacggttatccacagaatcaggggataacgcaggaaagaacatgtgagcaaaaggccagcaaaaggccaggaaccgtaaaaaggccgcgttgctggcgtttttccataggctccgcccccctgacgagcatcacaaaaatcgacgctcaagtcagaggtggcgaaacccgacaggactataaagataccaggcgtttccccctggaagctccctcgtgcgctctcctgttccgaccctgccgcttaccggatacctgtccgcctttctcccttcgggaagcgtggcgctttctcatagctcacgctgtaggtatctcagttcggtgtaggtcgttcgctccaagctgggctgtgtgcacgaaccccccgttcagcccgaccgctgcgccttatccggtaactatcgtcttgagtccaacccggtaagacacgacttatcgccactggcagcagccactggtaacaggattagcagagcgaggtatgtaggcggtgctacagagttcttgaagtggtggcctaactacggctacactagaaggacagtatttggtatctgcgctctgctgaagccagttaccttcggaaaaagagttggtagctcttgatccggcaaacaaaccaccgctggtagcggtggtttttttgtttgcaagcagcagattacgcgcagaaaaaaaggatctcaagaagatcctttgatcttttctacggggtctgacgctcagtggaacgaaaactcacgttaagggattttggtcatgagattatcaaaaaggatcttcacctagatccttttaaattaaaaatgaagttttaaatcaatctaaagtatatatgagtaaacttggtctgacagttaccaatgcttaatcagtgaggcacctatctcagcgatctgtctatttcgttcatccatagttgcctgactccccgtcgtgtagataactacgatacgggagggcttaccatctggccccagtgctgcaatgataccgcgagacccacgctcaccggctccagatttatcagcaataaaccagccagccggaagggccgagcgcagaagtggtcctgcaactttatccgcctccatccagtctattaattgttgccgggaagctagagtaagtagttcgccagttaatagtttgcgcaacgttgttgccattgctacaggcatcgtggtgtcacgctcgtcgtttggtatggcttcattcagctccggttcccaacgatcaaggcgagttacatgatcccccatgttgtgcaaaaaagcggttagctccttcggtcctccgatcgttgtcagaagtaagttggccgcagtgttatcactcatggttatggcagcactgcataattctcttactgtcatgccatccgtaagatgcttttctgtgactggtgagtactcaaccaagtcattctgagaatagtgtatgcggcgaccgagttgctcttgcccggcgtcaatacgggataataccgcgccacatagcagaactttaaaagtgctcatcattggaaaacgttcttcggggcgaaaactctcaaggatcttaccgctgttgagatccagttcgatgtaacccactcgtgcacccaactgatcttcagcatcttttactttcaccagcgtttctgggtgagcaaaaacaggaaggcaaaatgccgcaaaaaagggaataagggcgacacggaaatgttgaatactcatactcttcctttttcaatattattgaagcatttatcagggttattgtctcatgagcggatacatatttgaatgtatttagaaaaataaacaaataggggttccgcgcacatttccccgaaaagtgccacctaaattgta

SEQ ID NO: 18 - DNA, 1746 bp, synthetic construct
  source 1..1746: mol_type = other DNA
cccgcggctaagcgcgtgaagctggacgcccagcactccgactactccgacgacgagttctgtgccgacaagttgagcaactattcatgcgacagcgatctggagaacgcttccacctcggatgaggacagctcggacgacgaggtgatggtgcggcccaggacccttcgccgccggcggatctcctcctcttcttcagattccgaaagcgatattgagggcggtagggaggagtggtctcacgtagacaaccccccggttctggaggacttcctgggccaccagggcctgaacacggacgctgtgatcaataacattgaggatgctgtaaagctgttcatcggtgatgactttttcgagttcttggtggaggagtcgaatcgctactacaaccagaaccgcaacaacttcaaactatcaaagaagagcctgaaatggaaggacatcacccctcaggagatgaagaagttccttggtctcatcgtgctcatgggccaggtgcggaaagaccgcagggacgattattggaccacagaaccgtggacggagaccccctatttcgggaaaacaatgacgcgcgaccgcttccggcaaatttggaaggcctggcactttaacaacaacgcggacatcgtcaatgagagcgaccgcctctgtaaggtgcgccccgtcctggactacttcgtccctaagttcattaacatctacaagccccaccagcagctgtccttggatgagggcatcgtgccgtggagaggacgcctgtttttccgcgtgtacaatgcgggcaagattgtgaagtacggcatcctggtgcgcctgctgtgcgagtccgacaccggctacatctgcaacatggagatctattgcggggaggggaagcggctgctggagactatccagacggtggtgtccccatacaccgacagttggtaccatatatacatggataactactacaactccgtggccaattgcgaggccctgatgaaaaacaagttccgtatctgtggcaccattcgcaaaaaccgaggcatccctaaagacttccagaccatctctctgaagaaaggggagaccaagttcatccgcaagaacgacatcttactgcaggtctggcaaagtaagaagcccgtttacctaatctcgtccattcattctgcggagatggaagagtctcagaatattgaccgcacttctaagaagaagatcgttaagcctaacgcgctcattgactacaacaagcacatgaaaggtgtcgatcgcgcagaccagtacctctcgtattacagcatcctgcgtcgtaccgtgaaatggaccaagagattggccatgtatatgatcaactgcgccctgttcaacagctacgcggtgtacaagtcggtgcgccagcgcaagatgggctttaaaatgttcctgaagcagactgctatccactggctcactgatgacatacctgaagacatggatatcgtccccgacctgcagccggtgccctctacatccggaatgcgtgctaagccaccaacctccgacccgccatgtcgtctttccatggacatgagaaagcacactcttcaggccatcgtgggctccggcaagaagaagaatatcttacgccggtgccgagtctgtagcgtccacaagctgcgctccgagacccgctacatgtgcaagttttgtaacatccccctgcacaagggagcatgctttgagaagtaccataccctgaagaactacagccgt

SEQ ID NO: 19 - DNA, 6665 bp, synthetic construct
  source 1..6665: mol_type = other DNA
agcgttaatattttgttaaaattcgcgttaaatttttgttaaatcagctcattttttaaccaataggccgaaatcggcaaaatcccttataaatcaaaagaatagaccgagatagggttgagtgttgttccagtttggaacaagagtccactattaaagaacgtggactccaacgtcaaagggcgaaaaaccgtctatcagggcgatggcccactacgtgaaccatcaccctaatcaagttttttggggtcgaggtgccgtaaagcactaaatcggaaccctaaagggagcccccgatttagagcttgacggggaaagccggcgaacgtggcgagaaaggaagggaagaaagcgaaaggagcgggcgctagggcgctggcaagtgtagcggtcacgctgcgcgtaaccaccacacccgccgcgcttaatgcgccgctacagggcgcgtcccattcgccattcaggctgcgcaactgttgggaagggcgatcggtgcgggcctcttcgctattacgccagctggcgaaagggggatgtgctgcaaggcgattaagttgggtaacgccagggttttcccagtcacgacgttgtaaaacgacggccagtgaattgtaatacgactcactatagggcgaattgggtaccggccatgatggccgaattaattcaagctagtcgacattgattattgactagttattaatagtaatcaattacggggtcattagttcatagcccatatatggagttccgcgttacataacttacggtaaatggcccgcctggctgaccgcccaacgacccccgcccattgacgtcaataatgacgtatgttcccatagtaacgccaatagggactttccattgacgtcaatgggtggactatttacggtaaactgcccacttggcagtacatcaagtgtatcatatgccaagtacgccccctattgacgtcaatgacggtaaatggcccgcctggcattatgcccagtacatgaccttatgggactttcctacttggcagtacatctacgtattagtcatcgctattaccatgggtcgaggtgagccccacgttctgcttcactctccccatctcccccccctccccacccccaattttgtatttatttattttttaattattttgtgcagcgatgggggcggggggggggggggcgcgcgccaggcggggcggggcggggcgaggggcggggcggggcgaggcggagaggtgcggcggcagccaatcagagcggcgcgctccgaaagtttccttttatggcgaggcggcggcggcggcggccctataaaaagcgaagcgcgcggcgggcgggagtcgctgcgttgccttcgccccgtgccccgctccgcgccgcctcgcgccgcccgccccggctctgactgaccgcgttactcccacaggtgagcgggcgggacggcccttctcctccgggctgtaattagcgcttggtttaatgacggctcgtttcttttctgtggctgcgtgaaagccttaaagggctccgggagggccctttgtgcgggggggagcggctcggggggtgcgtgcgtgtgtgtgtgcgtggggagcgccgcgtgcggcccgcgctgcccggcggctgtgagcgctgcgggcgcggcgcggggctttgtgcgctccgcgtgtgcgcgaggggagcgcggccgggggcggtgccccgcggtgcgggggggctgcgaggggaacaaaggctgcgtgcggggtgtgtgcgtgggggggtgagcagggggtgtgggcgcggcggtcgggctgtaacccccccctgcacccccctccccgagttgctgagcacggcccggcttcgggtgcggggctccgtgcggggcgtggcgcggggctcgccgtgccgggcggggggtggcggcaggtgggggtgccgggcggggcggggccgcctcgggccggggagggctcgggggaggggcgcggcggccccggagcgccggcggctgtcgaggcgcggcgagccgcagccattgccttttatggtaatcgtgcgagagggcgcagggacttcctttgtcccaaatctggcggagccgaaatctgggaggcgccgccgcaccccctctagcgggcgcgggcgaagcggtgcggcgccggcaggaaggaaatgggcggggagggccttcgtgcgtcgccgcgccgccgtccccttctccatctccagcctcggggctgccgcagggggacggctgccttcgggggggacggggcagggcggggttcggcttctggcgtgtgaccggcggctctagagcctctgctaaccatgttcatgccttcttctttttcctacagctcctgggcaacgtgctggttattgtgctgtctcatcattttggcaaagaattggatccgccaccatgcccgcggctaagcgcgtgaagctggacgcccagcactccgactactccgacgacgagttctgtgccgacaagttgagcaactattcatgcgacagcgatctggagaacgcttccacctcggatgaggacagctcggacgacgaggtgatggtgcggcccaggacccttcgccgccggcggatctcctcctcttcttcagattccgaaagcgatattgagggcggtagggaggagtggtctcacgtagacaaccccccggttctggaggacttcctgggccaccagggcctgaacacggacgctgtgatcaataacattgaggatgctgtaaagctgttcatcggtgatgactttttcgagttcttggtggaggagtcgaatcgctactacaaccagaaccgcaacaacttcaaactatcaaagaagagcctgaaatggaaggacatcacccctcaggagatgaagaagttccttggtctcatcgtgctcatgggccaggtgcggaaagaccgcagggacgattattggaccacagaaccgtggacggagaccccctatttcgggaaaacaatgacgcgcgaccgcttccggcaaatttggaaggcctggcactttaacaacaacgcggacatcgtcaatgagagcgaccgcctctgtaaggtgcgccccgtcctggactacttcgtccctaagttcattaacatctacaagccccaccagcagctgtccttggatgagggcatcgtgccgtggagaggacgcctgtttttccgcgtgtacaatgcgggcaagattgtgaagtacggcatcctggtgcgcctgctgtgcgagtccgacaccggctacatctgcaacatggagatctattgcggggaggggaagcggctgctggagactatccagacggtggtgtccccatacaccgacagttggtaccatatatacatggataactactacaactccgtggccaattgcgaggccctgatgaaaaacaagttccgtatctgtggcaccattcgcaaaaaccgaggcatccctaaagacttccagaccatctctctgaagaaaggggagaccaagttcatccgcaagaacgacatcttactgcaggtctggcaaagtaagaagcccgtttacctaatctcgtccattcattctgcggagatggaagagtctcagaatattgaccgcacttctaagaagaagatcgttaagcctaacgcgctcattgactacaacaagcacatgaaaggtgtcgatcgcgcagaccagtacctctcgtattacagcatcctgcgtcgtaccgtgaaatggaccaagagattggccatgtatatgatcaactgcgccctgttcaacagctacgcggtgtacaagtcggtgcgccagcgcaagatgggctttaaaatgttcctgaagcagactgctatccactggctcactgatgacatacctgaagacatggatatcgtccccgacctgcagccggtgccctctacatccggaatgcgtgctaagccaccaacctccgacccgccatgtcgtctttccatggacatgagaaagcacactcttcaggccatcgtgggctccggcaagaagaagaatatcttacgccggtgccgagtctgtagcgtccacaagctgcgctccgagacccgctacatgtgcaagttttgtaacatccccctgcacaagggagcatgctttgagaagtaccataccctgaagaactacagccgttgactcgagggccgctgatcagcctcgactgtgccttctagttgccagccatctgttgtttgcccctcccccgtgccttccttgaccctggaaggtgccactcccactgtcctttcctaataaaatgaggaaattgcatcgcattgtctgagtaggtgtcattctattctggggggtggggtggggcaggacagcaagggggaggattgggaagacaatagcaggcatgctggggatgcggtgggctctatggcttctgaggcggaaagaaccagctggggcttaattaagagctccagcttttgttccctttagtgagggttaatttcgagcttggcgtaatcatggtcatagctgtttcctgtgtgaaattgttatccgctcacaattccacacaacatacgagccggaagcataaagtgtaaagcctggggtgcctaatgagtgagctaactcacattaattgcgttgcgctcactgcccgctttccagtcgggaaacctgtcgtgccagctgcattaatgaatcggccaacgcgcggggagaggcggtttgcgtattgggcgctcttccgcttcctcgctcactgactcgctgcgctcggtcgttcggctgcggcgagcggtatcagctcactcaaaggcggtaatacggttatccacagaatcaggggataacgcaggaaagaacatgtgagcaaaaggccagcaaaaggccaggaaccgtaaaaaggccgcgttgctggcgtttttccataggctccgcccccctgacgagcatcacaaaaatcgacgctcaagtcagaggtggcgaaacccgacaggactataaagataccaggcgtttccccctggaagctccctcgtgcgctctcctgttccgaccctgccgcttaccggatacctgtccgcctttctcccttcgggaagcgtggcgctttctcatagctcacgctgtaggtatctcagttcggtgtaggtcgttcgctccaagctgggctgtgtgcacgaaccccccgttcagcccgaccgctgcgccttatccggtaactatcgtcttgagtccaacccggtaagacacgacttatcgccactggcagcagccactggtaacaggattagcagagcgaggtatgtaggcggtgctacagagttcttgaagtggtggcctaactacggctacactagaaggacagtatttggtatctgcgctctgctgaagccagttaccttcggaaaaagagttggtagctcttgatccggcaaacaaaccaccgctggtagcggtggtttttttgtttgcaagcagcagattacgcgcagaaaaaaaggatctcaagaagatcctttgatcttttctacggggtctgacgctcagtggaacgaaaactcacgttaagggattttggtcatgagattatcaaaaaggatcttcacctagatccttttaaattaaaaatgaagttttaaatcaatctaaagtatatatgagtaaacttggtctgacagttaccaatgcttaatcagtgaggcacctatctcagcgatctgtctatttcgttcatccatagttgcctgactccccgtcgtgtagataactacgatacgggagggcttaccatctggccccagtgctgcaatgataccgcgagacccacgctcaccggctccagatttatcagcaataaaccagccagccggaagggccgagcgcagaagtggtcctgcaactttatccgcctccatccagtctattaattgttgccgggaagctagagtaagtagttcgccagttaatagtttgcgcaacgttgttgccattgctacaggcatcgtggtgtcacgctcgtcgtttggtatggcttcattcagctccggttcccaacgatcaaggcgagttacatgatcccccatgttgtgcaaaaaagcggttagctccttcggtcctccgatcgttgtcagaagtaagttggccgcagtgttatcactcatggttatggcagcactgcataattctcttactgtcatgccatccgtaagatgcttttctgtgactggtgagtactcaaccaagtcattctgagaatagtgtatgcggcgaccgagttgctcttgcccggcgtcaatacgggataataccgcgccacatagcagaactttaaaagtgctcatcattggaaaacgttcttcggggcgaaaactctcaaggatcttaccgctgttgagatccagttcgatgtaacccactcgtgcacccaactgatcttcagcatcttttactttcaccagcgtttctgggtgagcaaaaacaggaaggcaaaatgccgcaaaaaagggaataagggcgacacggaaatgttgaatactcatactcttcctttttcaatattattgaagcatttatcagggttattgtctcatgagcggatacatatttgaatgtatttagaaaaataaacaaataggggttccgcgcacatttccccgaaaagtgccacctaaattgta

SEQ ID NO: 20 - DNA, 1740 bp, synthetic construct
  source 1..1740: mol_type = other DNA
gcccagcactccgactactccgacgacgagttctgtgccgacaagttgagcaactattcatgcgacagcgatctggagaacgcttccacctcggatgaggacagctcggacgacgaggtgatggtgcggcccaggacccttcgccgccggcggatctcctcctcttcttcagattccgaaagcgatattgagggcggtagggaggagtggtctcacgtagacaaccccccggttctggaggacttcctgggccaccagggcctgaacacggacgctgtgatcaataacattgaggatgctgtaaagctgttcatcggtgatgactttttcgagttcttggtggaggagtcgaatcgctactacaaccagaaccgcaacaacttcaaactatcaaagaagagcctgaaatggaaggacatcacccctcaggagatgaagaagttccttggtctcatcgtgctcatgggccaggtgcggaaagaccgcagggacgattattggaccacagaaccgtggacggagaccccctatttcgggaaaacaatgacgcgcgaccgcttccggcaaatttggaaggcctggcactttaacaacaacgcggacatcgtcaatgagagcgaccgcctctgtaaggtgcgccccgtcctggactacttcgtccctaagttcattaacatctacaagccccaccagcagctgtccttggatgagggcatcgtgccgtggagaggacgcctgtttttccgcgtgtacaatgcgggcaagattgtgaagtacggcatcctggtgcgcctgctgtgcgagtccgacaccggctacatctgcaacatggagatctattgcggggaggggaagcggctgctggagactatccagacggtggtgtccccatacaccgacagttggtaccatatatacatggataactactacaactccgtggccaattgcgaggccctgatgaaaaacaagttccgtatctgtggcaccattcgcaaaaaccgaggcatccctaaagacttccagaccatctctctgaagaaaggggagaccaagttcatccgcaagaacgacatcttactgcaggtctggcaaagtaagaagcccgtttacctaatctcgtccattcattctgcggagatggaagagtctcagaatattgaccgcacttctaagaagaagatcgttaagcctaacgcgctcattgactacaacaagcacatgaaaggtgtcgatcgcgcagaccagtacctctcgtattacagcatcctgcgtcgtaccgtgaaatggaccaagagattggccatgtatatgatcaactgcgccctgttcaacagctacgcggtgtacaagtcggtgcgccagcgcaagatgggctttaaaatgttcctgaagcagactgctatccactggctcactgatgacatacctgaagacatggatatcgtccccgacctgcagccggtgccctctacatccggaatgcgtgctaagccaccaacctccgacccgccatgtcgtctttccatggacatgagaaagcacactcttcaggccatcgtgggctccggcaagaagaagaatatcttacgccggtgccgagtctgtagcgtccacaagctgcgctccgagacccgctacatgtgcaagttttgtaacatccccctgcacaagggagcatgctttgagaagtaccataccctgaagaactacagccgtcccaaaaagaagcgcaaggtg

SEQ ID NO: 21 - DNA, 6653 bp, synthetic construct
  source 1..6653: mol_type = other DNA
agcgttaatattttgttaaaattcgcgttaaatttttgttaaatcagctcattttttaaccaataggccgaaatcggcaaaatcccttataaatcaaaagaatagaccgagatagggttgagtgttgttccagtttggaacaagagtccactattaaagaacgtggactccaacgtcaaagggcgaaaaaccgtctatcagggcgatggcccactacgtgaaccatcaccctaatcaagttttttggggtcgaggtgccgtaaagcactaaatcggaaccctaaagggagcccccgatttagagcttgacggggaaagccggcgaacgtggcgagaaaggaagggaagaaagcgaaaggagcgggcgctagggcgctggcaagtgtagcggtcacgctgcgcgtaaccaccacacccgccgcgcttaatgcgccgctacagggcgcgtcccattcgccattcaggctgcgcaactgttgggaagggcgatcggtgcgggcctcttcgctattacgccagctggcgaaagggggatgtgctgcaaggcgattaagttgggtaacgccagggttttcccagtcacgacgttgtaaaacgacggccagtgaattgtaatacgactcactatagggcgaattgggtaccggccatgatggccgaattaattcaagctagtcgacattgattattgactagttattaatagtaatcaattacggggtcattagttcatagcccatatatggagttccgcgttacataacttacggtaaatggcccgcctggctgaccgcccaacgacccccgcccattgacgtcaataatgacgtatgttcccatagtaacgccaatagggactttccattgacgtcaatgggtggactatttacggtaaactgcccacttggcagtacatcaagtgtatcatatgccaagtacgccccctattgacgtcaatgacggtaaatggcccgcctggcattatgcccagtacatgaccttatgggactttcctacttggcagtacatctacgtattagtcatcgctattaccatgggtcgaggtgagccccacgttctgcttcactctccccatctcccccccctccccacccccaattttgtatttatttattttttaattattttgtgcagcgatgggggcggggggggggggggcgcgcgccaggcggggcggggcggggcgaggggcggggcggggcgaggcggagaggtgcggcggcagccaatcagagcggcgcgctccgaaagtttccttttatggcgaggcggcggcggcggcggccctataaaaagcgaagcgcgcggcgggcgggagtcgctgcgttgccttcgccccgtgccccgctccgcgccgcctcgcgccgcccgccccggctctgactgaccgcgttactcccacaggtgagcgggcgggacggcccttctcctccgggctgtaattagcgcttggtttaatgacggctcgtttcttttctgtggctgcgtgaaagccttaaagggctccgggagggccctttgtgcgggggggagcggctcggggggtgcgtgcgtgtgtgtgtgcgtggggagcgccgcgtgcggcccgcgctgcccggcggctgtgagcgctgcgggcgcggcgcggggctttgtgcgctccgcgtgtgcgcgaggggagcgcggccgggggcggtgccccgcggtgcgggggggctgcgaggggaacaaaggctgcgtgcggggtgtgtgcgtgggggggtgagcagggggtgtgggcgcggcggtcgggctgtaacccccccctgcacccccctccccgagttgctgagcacggcccggcttcgggtgcggggctccgtgcggggcgtggcgcggggctcgccgtgccgggcggggggtggcggcaggtgggggtgccgggcggggcggggccgcctcgggccggggagggctcgggggaggggcgcggcggccccggagcgccggcggctgtcgaggcgcggcgagccgcagccattgccttttatggtaatcgtgcgagagggcgcagggacttcctttgtcccaaatctggcggagccgaaatctgggaggcgccgccgcaccccctctagcgggcgcgggcgaagcggtgcggcgccggcaggaaggaaatgggcggggagggccttcgtgcgtcgccgcgccgccgtccccttctccatctccagcctcggggctgccgcagggggacggctgccttcgggggggacggggcagggcggggttcggcttctggcgtgtgaccggcggctctagagcctctgctaaccatgttcatgccttcttctttttcctacagctcctgggcaacgtgctggttattgtgctgtctcatcattttggcaaagaattggatccatggcccagcactccgactactccgacgacgagttctgtgccgacaagttgagcaactattcatgcgacagcgatctggagaacgcttccacctcggatgaggacagctcggacgacgaggtgatggtgcggcccaggacccttcgccgccggcggatctcctcctcttcttcagattccgaaagcgatattgagggcggtagggaggagtggtctcacgtagacaaccccccggttctggaggacttcctgggccaccagggcctgaacacggacgctgtgatcaataacattgaggatgctgtaaagctgttcatcggtgatgactttttcgagttcttggtggaggagtcgaatcgctactacaaccagaaccgcaacaacttcaaactatcaaagaagagcctgaaatggaaggacatcacccctcaggagatgaagaagttccttggtctcatcgtgctcatgggccaggtgcggaaagaccgcagggacgattattggaccacagaaccgtggacggagaccccctatttcgggaaaacaatgacgcgcgaccgcttccggcaaatttggaaggcctggcactttaacaacaacgcggacatcgtcaatgagagcgaccgcctctgtaaggtgcgccccgtcctggactacttcgtccctaagttcattaacatctacaagccccaccagcagctgtccttggatgagggcatcgtgccgtggagaggacgcctgtttttccgcgtgtacaatgcgggcaagattgtgaagtacggcatcctggtgcgcctgctgtgcgagtccgacaccggctacatctgcaacatggagatctattgcggggaggggaagcggctgctggagactatccagacggtggtgtccccatacaccgacagttggtaccatatatacatggataactactacaactccgtggccaattgcgaggccctgatgaaaaacaagttccgtatctgtggcaccattcgcaaaaaccgaggcatccctaaagacttccagaccatctctctgaagaaaggggagaccaagttcatccgcaagaacgacatcttactgcaggtctggcaaagtaagaagcccgtttacctaatctcgtccattcattctgcggagatggaagagtctcagaatattgaccgcacttctaagaagaagatcgttaagcctaacgcgctcattgactacaacaagcacatgaaaggtgtcgatcgcgcagaccagtacctctcgtattacagcatcctgcgtcgtaccgtgaaatggaccaagagattggccatgtatatgatcaactgcgccctgttcaacagctacgcggtgtacaagtcggtgcgccagcgcaagatgggctttaaaatgttcctgaagcagactgctatccactggctcactgatgacatacctgaagacatggatatcgtccccgacctgcagccggtgccctctacatccggaatgcgtgctaagccaccaacctccgacccgccatgtcgtctttccatggacatgagaaagcacactcttcaggccatcgtgggctccggcaagaagaagaatatcttacgccggtgccgagtctgtagcgtccacaagctgcgctccgagacccgctacatgtgcaagttttgtaacatccccctgcacaagggagcatgctttgagaagtaccataccctgaagaactacagccgtcccaaaaagaagcgcaaggtgtgactcgagggccgctgatcagcctcgactgtgccttctagttgccagccatctgttgtttgcccctcccccgtgccttccttgaccctggaaggtgccactcccactgtcctttcctaataaaatgaggaaattgcatcgcattgtctgagtaggtgtcattctattctggggggtggggtggggcaggacagcaagggggaggattgggaagacaatagcaggcatgctggggatgcggtgggctctatggcttctgaggcggaaagaaccagctggggcttaattaagagctccagcttttgttccctttagtgagggttaatttcgagcttggcgtaatcatggtcatagctgtttcctgtgtgaaattgttatccgctcacaattccacacaacatacgagccggaagcataaagtgtaaagcctggggtgcctaatgagtgagctaactcacattaattgcgttgcgctcactgcccgctttccagtcgggaaacctgtcgtgccagctgcattaatgaatcggccaacgcgcggggagaggcggtttgcgtattgggcgctcttccgcttcctcgctcactgactcgctgcgctcggtcgttcggctgcggcgagcggtatcagctcactcaaaggcggtaatacggttatccacagaatcaggggataacgcaggaaagaacatgtgagcaaaaggccagcaaaaggccaggaaccgtaaaaaggccgcgttgctggcgtttttccataggctccgcccccctgacgagcatcacaaaaatcgacgctcaagtcagaggtggcgaaacccgacaggactataaagataccaggcgtttccccctggaagctccctcgtgcgctctcctgttccgaccctgccgcttaccggatacctgtccgcctttctcccttcgggaagcgtggcgctttctcatagctcacgctgtaggtatctcagttcggtgtaggtcgttcgctccaagctgggctgtgtgcacgaaccccccgttcagcccgaccgctgcgccttatccggtaactatcgtcttgagtccaacccggtaagacacgacttatcgccactggcagcagccactggtaacaggattagcagagcgaggtatgtaggcggtgctacagagttcttgaagtggtggcctaactacggctacactagaaggacagtatttggtatctgcgctctgctgaagccagttaccttcggaaaaagagttggtagctcttgatccggcaaacaaaccaccgctggtagcggtggtttttttgtttgcaagcagcagattacgcgcagaaaaaaaggatctcaagaagatcctttgatcttttctacggggtctgacgctcagtggaacgaaaactcacgttaagggattttggtcatgagattatcaaaaaggatcttcacctagatccttttaaattaaaaatgaagttttaaatcaatctaaagtatatatgagtaaacttggtctgacagttaccaatgcttaatcagtgaggcacctatctcagcgatctgtctatttcgttcatccatagttgcctgactccccgtcgtgtagataactacgatacgggagggcttaccatctggccccagtgctgcaatgataccgcgagacccacgctcaccggctccagatttatcagcaataaaccagccagccggaagggccgagcgcagaagtggtcctgcaactttatccgcctccatccagtctattaattgttgccgggaagctagagtaagtagttcgccagttaatagtttgcgcaacgttgttgccattgctacaggcatcgtggtgtcacgctcgtcgtttggtatggcttcattcagctccggttcccaacgatcaaggcgagttacatgatcccccatgttgtgcaaaaaagcggttagctccttcggtcctccgatcgttgtcagaagtaagttggccgcagtgttatcactcatggttatggcagcactgcataattctcttactgtcatgccatccgtaagatgcttttctgtgactggtgagtactcaaccaagtcattctgagaatagtgtatgcggcgaccgagttgctcttgcccggcgtcaatacgggataataccgcgccacatagcagaactttaaaagtgctcatcattggaaaacgttcttcggggcgaaaactctcaaggatcttaccgctgttgagatccagttcgatgtaacccactcgtgcacccaactgatcttcagcatcttttactttcaccagcgtttctgggtgagcaaaaacaggaaggcaaaatgccgcaaaaaagggaataagggcgacacggaaatgttgaatactcatactcttcctttttcaatattattgaagcatttatcagggttattgtctcatgagcggatacatatttgaatgtatttagaaaaataaacaaataggggttccgcgcacatttccccgaaaagtgccacctaaattgta

SEQ ID NO: 22 - DNA, 1746 bp, synthetic construct
  source 1..1746: mol_type = other DNA
gcccagcactccgactactccgacgacgagttctgtgccgacaagttgagcaactattcatgcgacagcgatctggagaacgcttccacctcggatgaggacagctcggacgacgaggtgatggtgcggcccaggacccttcgccgccggcggatctcctcctcttcttcagattccgaaagcgatattgagggcggtagggaggagtggtctcacgtagacaaccccccggttctggaggacttcctgggccaccagggcctgaacacggacgctgtgatcaataacattgaggatgctgtaaagctgttcatcggtgatgactttttcgagttcttggtggaggagtcgaatcgctactacaaccagaaccgcaacaacttcaaactatcaaagaagagcctgaaatggaaggacatcacccctcaggagatgaagaagttccttggtctcatcgtgctcatgggccaggtgcggaaagaccgcagggacgattattggaccacagaaccgtggacggagaccccctatttcgggaaaacaatgacgcgcgaccgcttccggcaaatttggaaggcctggcactttaacaacaacgcggacatcgtcaatgagagcgaccgcctctgtaaggtgcgccccgtcctggactacttcgtccctaagttcattaacatctacaagccccaccagcagctgtccttggatgagggcatcgtgccgtggagaggacgcctgtttttccgcgtgtacaatgcgggcaagattgtgaagtacggcatcctggtgcgcctgctgtgcgagtccgacaccggctacatctgcaacatggagatctattgcggggaggggaagcggctgctggagactatccagacggtggtgtccccatacaccgacagttggtaccatatatacatggataactactacaactccgtggccaattgcgaggccctgatgaaaaacaagttccgtatctgtggcaccattcgcaaaaaccgaggcatccctaaagacttccagaccatctctctgaagaaaggggagaccaagttcatccgcaagaacgacatcttactgcaggtctggcaaagtaagaagcccgtttacctaatctcgtccattcattctgcggagatggaagagtctcagaatattgaccgcacttctaagaagaagatcgttaagcctaacgcgctcattgactacaacaagcacatgaaaggtgtcgatcgcgcagaccagtacctctcgtattacagcatcctgcgtcgtaccgtgaaatggaccaagagattggccatgtatatgatcaactgcgccctgttcaacagctacgcggtgtacaagtcggtgcgccagcgcaagatgggctttaaaatgttcctgaagcagactgctatccactggctcactgatgacatacctgaagacatggatatcgtccccgacctgcagccggtgccctctacatccggaatgcgtgctaagccaccaacctccgacccgccatgtcgtctttccatggacatgagaaagcacactcttcaggccatcgtgggctccggcaagaagaagaatatcttacgccggtgccgagtctgtagcgtccacaagctgcgctccgagacccgctacatgtgcaagttttgtaacatccccctgcacaagggagcatgctttgagaagtaccataccctgaagaactacagccgtcccgcggctaagcgcgtgaagctggac

SEQ ID NO: 23 - DNA, 6659 bp, synthetic construct
  source 1..6659: mol_type = other DNA
agcgttaatattttgttaaaattcgcgttaaatttttgttaaatcagctcattttttaaccaataggccgaaatcggcaaaatcccttataaatcaaaagaatagaccgagatagggttgagtgttgttccagtttggaacaagagtccactattaaagaacgtggactccaacgtcaaagggcgaaaaaccgtctatcagggcgatggcccactacgtgaaccatcaccctaatcaagttttttggggtcgaggtgccgtaaagcactaaatcggaaccctaaagggagcccccgatttagagcttgacggggaaagccggcgaacgtggcgagaaaggaagggaagaaagcgaaaggagcgggcgctagggcgctggcaagtgtagcggtcacgctgcgcgtaaccaccacacccgccgcgcttaatgcgccgctacagggcgcgtcccattcgccattcaggctgcgcaactgttgggaagggcgatcggtgcgggcctcttcgctattacgccagctggcgaaagggggatgtgctgcaaggcgattaagttgggtaacgccagggttttcccagtcacgacgttgtaaaacgacggccagtgaattgtaatacgactcactatagggcgaattgggtaccggccatgatggccgaattaattcaagctagtcgacattgattattgactagttattaatagtaatcaattacggggtcattagttcatagcccatatatggagttccgcgttacataacttacggtaaatggcccgcctggctgaccgcccaacgacccccgcccattgacgtcaataatgacgtatgttcccatagtaacgccaatagggactttccattgacgtcaatgggtggactatttacggtaaactgcccacttggcagtacatcaagtgtatcatatgccaagtacgccccctattgacgtcaatgacggtaaatggcccgcctggcattatgcccagtacatgaccttatgggactttcctacttggcagtacatctacgtattagtcatcgctattaccatgggtcgaggtgagccccacgttctgcttcactctccccatctcccccccctccccacccccaattttgtatttatttattttttaattattttgtgcagcgatgggggcggggggggggggggcgcgcgccaggcggggcggggcggggcgaggggcggggcggggcgaggcggagaggtgcggcggcagccaatcagagcggcgcgctccgaaagtttccttttatggcgaggcggcggcggcggcggccctataaaaagcgaagcgcgcggcgggcgggagtcgctgcgttgccttcgccccgtgccccgctccgcgccgcctcgcgccgcccgccccggctctgactgaccgcgttactcccacaggtgagcgggcgggacggcccttctcctccgggctgtaattagcgcttggtttaatgacggctcgtttcttttctgtggctgcgtgaaagccttaaagggctccgggagggccctttgtgcgggggggagcggctcggggggtgcgtgcgtgtgtgtgtgcgtggggagcgccgcgtgcggcccgcgctgcccggcggctgtgagcgctgcgggcgcggcgcggggctttgtgcgctccgcgtgtgcgcgaggggagcgcggccgggggcggtgccccgcggtgcgggggggctgcgaggggaacaaaggctgcgtgcggggtgtgtgcgtgggggggtgagcagggggtgtgggcgcggcggtcgggctgtaacccccccctgcacccccctccccgagttgctgagcacggcccggcttcgggtgcggggctccgtgcggggcgtggcgcggggctcgccgtgccgggcggggggtggcggcaggtgggggtgccgggcggggcggggccgcctcgggccggggagggctcgggggaggggcgcggcggccccggagcgccggcggctgtcgaggcgcggcgagccgcagccattgccttttatggtaatcgtgcgagagggcgcagggacttcctttgtcccaaatctggcggagccgaaatctgggaggcgccgccgcaccccctctagcgggcgcgggcgaagcggtgcggcgccggcaggaaggaaatgggcggggagggccttcgtgcgtcgccgcgccgccgtccccttctccatctccagcctcggggctgccgcagggggacggctgccttcgggggggacggggcagggcggggttcggcttctggcgtgtgaccggcggctctagagcctctgctaaccatgttcatgccttcttctttttcctacagctcctgggcaacgtgctggttattgtgctgtctcatcattttggcaaagaattggatccatggcccagcactccgactactccgacgacgagttctgtgccgacaagttgagcaactattcatgcgacagcgatctggagaacgcttccacctcggatgaggacagctcggacgacgaggtgatggtgcggcccaggacccttcgccgccggcggatctcctcctcttcttcagattccgaaagcgatattgagggcggtagggaggagtggtctcacgtagacaaccccccggttctggaggacttcctgggccaccagggcctgaacacggacgctgtgatcaataacattgaggatgctgtaaagctgttcatcggtgatgactttttcgagttcttggtggaggagtcgaatcgctactacaaccagaaccgcaacaacttcaaactatcaaagaagagcctgaaatggaaggacatcacccctcaggagatgaagaagttccttggtctcatcgtgctcatgggccaggtgcggaaagaccgcagggacgattattggaccacagaaccgtggacggagaccccctatttcgggaaaacaatgacgcgcgaccgcttccggcaaatttggaaggcctggcactttaacaacaacgcggacatcgtcaatgagagcgaccgcctctgtaaggtgcgccccgtcctggactacttcgtccctaagttcattaacatctacaagccccaccagcagctgtccttggatgagggcatcgtgccgtggagaggacgcctgtttttccgcgtgtacaatgcgggcaagattgtgaagtacggcatcctggtgcgcctgctgtgcgagtccgacaccggctacatctgcaacatggagatctattgcggggaggggaagcggctgctggagactatccagacggtggtgtccccatacaccgacagttggtaccatatatacatggataactactacaactccgtggccaattgcgaggccctgatgaaaaacaagttccgtatctgtggcaccattcgcaaaaaccgaggcatccctaaagacttccagaccatctctctgaagaaaggggagaccaagttcatccgcaagaacgacatcttactgcaggtctggcaaagtaagaagcccgtttacctaatctcgtccattcattctgcggagatggaagagtctcagaatattgaccgcacttctaagaagaagatcgttaagcctaacgcgctcattgactacaacaagcacatgaaaggtgtcgatcgcgcagaccagtacctctcgtattacagcatcctgcgtcgtaccgtgaaatggaccaagagattggccatgtatatgatcaactgcgccctgttcaacagctacgcggtgtacaagtcggtgcgccagcgcaagatgggctttaaaatgttcctgaagcagactgctatccactggctcactgatgacatacctgaagacatggatatcgtccccgacctgcagccggtgccctctacatccggaatgcgtgctaagccaccaacctccgacccgccatgtcgtctttccatggacatgagaaagcacactcttcaggccatcgtgggctccggcaagaagaagaatatcttacgccggtgccgagtctgtagcgtccacaagctgcgctccgagacccgctacatgtgcaagttttgtaacatccccctgcacaagggagcatgctttgagaagtaccataccctgaagaactacagccgtcccgcggctaagcgcgtgaagctggactgactcgagggccgctgatcagcctcgactgtgccttctagttgccagccatctgttgtttgcccctcccccgtgccttccttgaccctggaaggtgccactcccactgtcctttcctaataaaatgaggaaattgcatcgcattgtctgagtaggtgtcattctattctggggggtggggtggggcaggacagcaagggggaggattgggaagacaatagcaggcatgctggggatgcggtgggctctatggcttctgaggcggaaagaaccagctggggcttaattaagagctccagcttttgttccctttagtgagggttaatttcgagcttggcgtaatcatggtcatagctgtttcctgtgtgaaattgttatccgctcacaattccacacaacatacgagccggaagcataaagtgtaaagcctggggtgcctaatgagtgagctaactcacattaattgcgttgcgctcactgcccgctttccagtcgggaaacctgtcgtgccagctgcattaatgaatcggccaacgcgcggggagaggcggtttgcgtattgggcgctcttccgcttcctcgctcactgactcgctgcgctcggtcgttcggctgcggcgagcggtatcagctcactcaaaggcggtaatacggttatccacagaatcaggggataacgcaggaaagaacatgtgagcaaaaggccagcaaaaggccaggaaccgtaaaaaggccgcgttgctggcgtttttccataggctccgcccccctgacgagcatcacaaaaatcgacgctcaagtcagaggtggcgaaacccgacaggactataaagataccaggcgtttccccctggaagctccctcgtgcgctctcctgttccgaccctgccgcttaccggatacctgtccgcctttctcccttcgggaagcgtggcgctttctcatagctcacgctgtaggtatctcagttcggtgtaggtcgttcgctccaagctgggctgtgtgcacgaaccccccgttcagcccgaccgctgcgccttatccggtaactatcgtcttgagtccaacccggtaagacacgacttatcgccactggcagcagccactggtaacaggattagcagagcgaggtatgtaggcggtgctacagagttcttgaagtggtggcctaactacggctacactagaaggacagtatttggtatctgcgctctgctgaagccagttaccttcggaaaaagagttggtagctcttgatccggcaaacaaaccaccgctggtagcggtggtttttttgtttgcaagcagcagattacgcgcagaaaaaaaggatctcaagaagatcctttgatcttttctacggggtctgacgctcagtggaacgaaaactcacgttaagggattttggtcatgagattatcaaaaaggatcttcacctagatccttttaaattaaaaatgaagttttaaatcaatctaaagtatatatgagtaaacttggtctgacagttaccaatgcttaatcagtgaggcacctatctcagcgatctgtctatttcgttcatccatagttgcctgactccccgtcgtgtagataactacgatacgggagggcttaccatctggccccagtgctgcaatgataccgcgagacccacgctcaccggctccagatttatcagcaataaaccagccagccggaagggccgagcgcagaagtggtcctgcaactttatccgcctccatccagtctattaattgttgccgggaagctagagtaagtagttcgccagttaatagtttgcgcaacgttgttgccattgctacaggcatcgtggtgtcacgctcgtcgtttggtatggcttcattcagctccggttcccaacgatcaaggcgagttacatgatcccccatgttgtgcaaaaaagcggttagctccttcggtcctccgatcgttgtcagaagtaagttggccgcagtgttatcactcatggttatggcagcactgcataattctcttactgtcatgccatccgtaagatgcttttctgtgactggtgagtactcaaccaagtcattctgagaatagtgtatgcggcgaccgagttgctcttgcccggcgtcaatacgggataataccgcgccacatagcagaactttaaaagtgctcatcattggaaaacgttcttcggggcgaaaactctcaaggatcttaccgctgttgagatccagttcgatgtaacccactcgtgcacccaactgatcttcagcatcttttactttcaccagcgtttctgggtgagcaaaaacaggaaggcaaaatgccgcaaaaaagggaataagggcgacacggaaatgttgaatactcatactcttcctttttcaatattattgaagcatttatcagggttattgtctcatgagcggatacatatttgaatgtatttagaaaaataaacaaataggggttccgcgcacatttccccgaaaagtgccacctaaattgta